European Patent Application EP 4 413 995 A1, published August 14, 2024. Title: ANTI-CD123 CHIMERIC ANTIGEN RECEPTORS T CELLS FOR USE IN THE TREATEMENT OF AUTOIMMUNE DISEASES. Applicant: UNIVERSITÉ FRANCHE-COMTÉ. Application EP. The sequence listing filed with the application follows.

SEQUENCE LISTING (6 sequences)

SEQ ID NO: 1 - protein, 9 aa, Mus
GYSITSDYT

SEQ ID NO: 2 - protein, 7 aa, Mus
ISFSGST

SEQ ID NO: 3 - protein, 6 aa, Mus
ARGLDY

SEQ ID NO: 4 - protein, 7 aa, Mus
SSISSSY

SEQ ID NO: 5 - protein, 9 aa, Mus
HQLHRSPWT

SEQ ID NO: 6 - DNA, 1533 bp, Homo sapiens
  source 1..1533: mol_type = other DNA
atgaaactgcccgtgagactgctggtgctgatgttttggattcccgcttcctcgagcgacccatacgatgttccagattacgccatcctgtctgatgtgcagcttcaggagtcgggacctggcctggtgaaaccttctcagtctctgtccctcacctgcactgtcactggctactcaatcaccagtgattatacctggaactggattcggcagtttccaggaaacaaactggagtggatgggctacataagcttcagtggtagcactagctacaacccatctctcaaaagtcgactctctatcacccgagacacatccaagaaccagttcttcctgcagttgaattctgtgactactgaggacacagccacatattactgtgcaagagggctcgactactggggccaaggcaccactctcacagtctcctcaggaggcggttcaggcggaggtggctctggcggtggcggatcgataatgtccagaggacaaattgttctcacccagtctccagcaatcatgtctgcatctcttggggaacgggtcaccatgacctgcactgccagctcaagtataagttccagttacttgtactggtaccagcagaagccaggctcctcccccaaactctggatttatagcacatccaacctggcttctggagtcccagctcgcttcagtggcagtgggtctgggacctcttactctctcacaatcagcagcatggaggctgaagatgctgccacttattactgccaccagttgcatcgttccccgtggacgttcggtggaggcaccaagctggaaatcaaagagcccaaatcttgtgacaaaactcacacatgcccaccgtgccctgatcccaaattttgggtgctggtggtggttggtggagtcctggcttgctatagcttgctagtaacagtggcctttattattttctgggtgaggagtaagaggagcaggctcctgcacagtgactacatgaacatgactccccgccgccccgggcccacccgcaagcattaccagccctatgccccaccacgcgacttcgcagcctatcgctccaaacggggcagaaagaaactcctgtatatattcaaacaaccatttatgagaccagtacaaactactcaagaggaagatggctgtagctgccgatttccagaagaagaagaaggaggatgtgaactgagagtgaagttcagcaggagcgcagacgcccccgcgtaccagcagggccagaaccagctctataacgagctcaatctaggacgaagagaggagtacgatgttttggacaagaggcgtggccgggaccctgagatggggggaaagccgagaaggaagaaccctcaggaaggcctgtacaatgaactgcagaaagataagatggcggaggcctacagtgagattgggatgaaaggcgagcgccggaggggcaaggggcacgatggcctttaccagggtctcagtacagccaccaaggacacctacgacgcccttcacatgcaggccctgccccctcgc